European Patent Specification EP 4 240 328 B1, published April 22, 2026. Title: Liposom, zw³aszcza do stosowania w leczeniu COVID-19. Applicant: Acellmed Sp. z o.o. The sequence listing filed with the application follows.

SEQUENCE LISTING (3 sequences)

SEQ ID NO: 1 - protein, 24 aa, artificial
  peptyd 1
EEQAKTFLDKFNHEAEDLFYQSSC

SEQ ID NO: 2 - protein, 8 aa, artificial
  peptyd 2
LGKGDFRC

SEQ ID NO: 3 - protein, 32 aa, artificial
  peptyd 3
EEQAKTFLDKFNHEAEDLFYQSSGLGKGDFRC